European Patent Application EP 4 516 928 A1, published March 5, 2025. Title: Composition for determining whether a nucleic acid is methylated and Method for determining whether a nucleic acid is methylated. Applicant: UIF (University Industry Foundation), Yonsei University. The sequence listing filed with the application follows.

SEQUENCE LISTING (11 sequences)

SEQ ID NO: 1 - DNA, 480 bp, synthetic construct
  misc_feature 1..480: note = Nucleic acid to be identified
  source 1..480: mol_type = other DNA
aggaaggagacggggtggcgccaaggaaggaggagaaaaggcggccgagaaaaggaggagggcaaggggaagaggaagggcgagggaggagcctgaggagactcgcccggctcaaccccgacgtccgcgccccggccgcctgttggccatggcgggcctgggcctgggctccgccgttcccgtgtggctggccgaggacgacctcggctgcatcatctgccaggggctgctggactggcccgccacgctgccctgcggccacagcttctgccgccactgcctggaggccctgtggggcgcccgcgacgcccgccgctgggcctgccccacttgccgccagggcgccgcgcagcagccgcacctgcggaagaacacgctactgcaggacctggccgacaagtaccgccgcgccgcacgcgagatacaggcgggctccgaccctgcccactgcccctgcccgggctccagttccctctccag

SEQ ID NO: 2 - DNA, 480 bp, synthetic construct
  misc_feature 1..480: note = Methylated nucleic acid to be identified treated with sulfite
  source 1..480: mol_type = other DNA
aggaaggagacggggtggcgttaaggaaggaggagaaaaggcggtcgagaaaaggaggagggtaaggggaagaggaagggcgagggaggagtttgaggagattcgttcggtttaatttcgacgttcgcgtttcggtcgtttgttggttatggcgggtttgggtttgggtttcgtcgttttcgtgtggttggtcgaggacgatttcggttgtattatttgttaggggttgttggattggttcgttacgttgttttgcggttatagtttttgtcgttattgtttggaggttttgtggggcgttcgcgacgttcgtcgttgggtttgttttatttgtcgttagggcgtcgcgtagtagtcgtatttgcggaagaatacgttattgtaggatttggtcgataagtatcgtcgcgtcgtacgcgagatataggcgggtttcgattttgtttattgtttttgttcgggttttagttttttttttag

SEQ ID NO: 3 - DNA, 480 bp, synthetic construct
  misc_feature 1..480: note = Unmethylated nucleic acid to be identified treated with sulfite
  source 1..480: mol_type = other DNA
aggaaggagatggggtggtgttaaggaaggaggagaaaaggtggttgagaaaaggaggagggtaaggggaagaggaagggtgagggaggagtttgaggagatttgtttggtttaattttgatgtttgtgttttggttgtttgttggttatggtgggtttgggtttgggttttgttgtttttgtgtggttggttgaggatgattttggttgtattatttgttaggggttgttggattggtttgttatgttgttttgtggttatagtttttgttgttattgtttggaggttttgtggggtgtttgtgatgtttgttgttgggtttgttttatttgttgttagggtgttgtgtagtagttgtatttgtggaagaatatgttattgtaggatttggttgataagtattgttgtgttgtatgtgagatataggtgggttttgattttgtttattgtttttgtttgggttttagttttttttttag

SEQ ID NO: 4 - DNA, 25 bp, synthetic construct
  misc_feature 1..25: note = Methylation primer FWD
  source 1..25: mol_type = other DNA
ttatggcgggtttgggtttgggttt

SEQ ID NO: 5 - DNA, 25 bp, synthetic construct
  misc_feature 1..25: note = Unmethylation primer FWD
  source 1..25: mol_type = other DNA
ttatggtgggtttgggtttgggttt

SEQ ID NO: 6 - DNA, 24 bp, synthetic construct
  misc_feature 1..24: note = common REV primer
  source 1..24: mol_type = other DNA
caacccctaacaaataatacaacc

SEQ ID NO: 7 - DNA, 24 bp, synthetic construct
  misc_feature 1..24: note = methylation independent primer FWD
  source 1..24: mol_type = other DNA
gttgtattatttgttaggggttgt

SEQ ID NO: 8 - DNA, 22 bp, synthetic construct
  misc_feature 1..22: note = methylation independent primer RVS
  source 1..22: mol_type = other DNA
ccacaaaacctccaaacaataa

SEQ ID NO: 9 - DNA, 26 bp, synthetic construct
  misc_feature 1..26: note = primer with CpG recognition site FWD
  source 1..26: mol_type = other DNA
tttcggttgtattatttgttaggggt

SEQ ID NO: 10 - DNA, 22 bp, synthetic construct
  misc_feature 1..22: note = primer with CpG recognition site RVS
  source 1..22: mol_type = other DNA
aacgccccacaaaacctccaaa

SEQ ID NO: 11 - DNA, 18 bp, synthetic construct
  misc_feature 1..18: note = Fluorescent probe
  source 1..18: mol_type = other DNA
ggttcgttacgttgtttt